European Patent Specification EP 3 725 879 B1, published July 3, 2024. Title: Genetically modified non-human model animals. Applicant: Iori Ohmori Mamoru Ouchida Tomoji Mashimo. The sequence listing filed with the application follows.

SEQUENCE LISTING (41 sequences)

SEQ ID NO: 1 - DNA, 318 bp, Rattus norvegicus
atggtgaagctgatcgagagcaaggaagcttttcaggaggccctggccgctgcgggagacaagcttgtggtagtggacttctctgccacgtggtgtggaccttgcaaaatgatcaagcccttctttcattccctctgtgacaagtattccaatgtggtgttccttgaagtagacgtggatgactgccaggatgttgctgcagactgtgaagtcaaatgcatgccgaccttccagttctataaaaagggtcaaaaggttggggagttctctggtgctaacaaggaaaagctcgaagccactattacggagtttgcctaa

SEQ ID NO: 2 - protein, 105 aa, Rattus norvegicus
MVKLIESKEAFQEALAAAGDKLVVVDFSATWCGPCKMIKPFFHSLCDKYSNVVFLEVDVDDCQDVAADCEVKCMPTFQFYKKGQKVGEFSGANKEKLEATITEFA

SEQ ID NO: 3 - protein, 19 aa, Rattus norvegicus
KYSNVVFLEVDVDDCQDVA

SEQ ID NO: 4 - protein, 19 aa, Mus musculus
KYSNVVFLEVDVDDCQDVA

SEQ ID NO: 5 - protein, 19 aa, Nannospalax Galili
KYSNVVFLEVDVDDCQDVA

SEQ ID NO: 6 - protein, 19 aa, Carlito Syrichta
KYSNVVFLEVDVDDCQDVA

SEQ ID NO: 7 - protein, 19 aa, Peromyscus maniculatus
KYSNVVFLEVDVDDCQDVA

SEQ ID NO: 8 - protein, 19 aa, Bos mutus
KYSNVVFLEVDVDDCQDVA

SEQ ID NO: 9 - protein, 19 aa, Ovis aries
KYSNVVFLEVDVDDCQDVA

SEQ ID NO: 10 - protein, 19 aa, Pteropus alecto
KYSNVVFLEVDVDDCQDVA

SEQ ID NO: 11 - protein, 19 aa, Rousettus aegyptiacus
KYSNVVFLEVDVDDCQDVA

SEQ ID NO: 12 - protein, 19 aa, Galeopterus Variegatus
KYSNVVFLEVDVDDCQDVA

SEQ ID NO: 13 - protein, 19 aa, Vicugna Pacos
KYSNVVFLEVDVDDCQDVA

SEQ ID NO: 14 - protein, 19 aa, Odobenus Rosmarus Divergens
KYSNVVFLEVDVDDCQDVA

SEQ ID NO: 15 - protein, 19 aa, Acinonyx jubatus
KYSNVVFLEVDVDDCQDVA

SEQ ID NO: 16 - protein, 19 aa, Mustela Putorius Furo
KYSNVVFLEVDVDDCQDVA

SEQ ID NO: 17 - protein, 19 aa, Balaenoptera Acutorostrata Sca
KYSNVVFLEVDVDDCQDVA

SEQ ID NO: 18 - protein, 19 aa, Sus scrofa
KYSNVVFLEVDVDDCQDVA

SEQ ID NO: 19 - protein, 19 aa, Macaca mulatta
KYSNVVFLEVDVDDCQDVA

SEQ ID NO: 20 - protein, 19 aa, Colobus angolensis
KYSNVVFLEVDVDDCQDVA

SEQ ID NO: 21 - protein, 19 aa, Ceratotherium simum
KYSNVVFLEVDVDDCQDVA

SEQ ID NO: 22 - protein, 19 aa, Callithrix jacchus
KYSNVVFLEVDVDDCQDVA

SEQ ID NO: 23 - protein, 19 aa, Propithecus sp.
KYSNVVFLEVDVDDCQDVA

SEQ ID NO: 24 - protein, 19 aa, Camelus sp.
KYSNVVFLEVDVDDCQDVA

SEQ ID NO: 25 - protein, 19 aa, Manis javanica
KYSNVVFLEVDVDDCQDVA

SEQ ID NO: 26 - protein, 19 aa, Ursus sp.
KYSNVVFLEVDVDDCQDVA

SEQ ID NO: 27 - protein, 19 aa, Miniopterus Natalensis
KYSNVVFLEVDVDDCQDVA

SEQ ID NO: 28 - protein, 19 aa, Cavia porcellus
KYSNVVFLEVDVDDCQDVA

SEQ ID NO: 29 - protein, 19 aa, Aotus nancymaae
KYSNVVFLEVDVDDCQDVA

SEQ ID NO: 30 - protein, 19 aa, Tursiops truncatus
KYSNVVFLEVDVDDCQDVA

SEQ ID NO: 31 - protein, 19 aa, Ailuropoda melanoleuca
KYSNVVFLEVDVDDCQDVA

SEQ ID NO: 32 - protein, 19 aa, Equus caballus
KYSNVVFLEVDVDDCQDVA

SEQ ID NO: 33 - protein, 19 aa, Bos taurus
KYSNVVFLEVDVDDCQDVA

SEQ ID NO: 34 - protein, 19 aa, Acinetobacter sp.
KYSNVIFLEVDVDDCQDVA

SEQ ID NO: 35 - protein, 19 aa, Homo sapiens
KYSNVIFLEVDVDDCQDVA

SEQ ID NO: 36 - protein, 19 aa, Nomascus Leucogenys
KYSNVIFLEVDVDDCQDVA

SEQ ID NO: 37 - protein, 19 aa, Octodon degus
KYSNVLFLEVDVDDCQDVA

SEQ ID NO: 38 - protein, 19 aa, Ictidomys Tridecemlineatus
KYSNVLFLEVDVDDCQDVA

SEQ ID NO: 39 - protein, 19 aa, Marmota marmota
KYSNVLFLEVDVDDCQDVA

SEQ ID NO: 40 - protein, 19 aa, Chinchilla laniger
KYSNVLFLEVDVDDCQDVA

SEQ ID NO: 41 - protein, 19 aa, Eptesicus fuscus
KYSNVLFLEVDVDDCQDVA